European Patent Specification EP 3 475 443 B1, published February 12, 2025. Title: METHODS AND COMPOSITIONS FOR DETECTING OR MEASURING CASPASES OR APOPTOSIS. Applicant: LIFE TECHNOLOGIES CORPORATION. The sequence listing filed with the application follows.

SEQUENCE LISTING (24 sequences)

SEQ ID NO: 1 - protein, 4 aa, Artificial Sequence
  source: /note="Description of Artificial Sequence: Synthetic peptide with caspase recognition/cleavage sequence, e.g., for Caspase 3/7"
DEVD

SEQ ID NO: 2 - protein, 4 aa, Artificial Sequence
  source: /note="Description of Artificial Sequence: Synthetic peptide with caspase recognition/cleavage sequence, e.g., for Caspase 9"
LEHD

SEQ ID NO: 3 - protein, 5 aa, Artificial Sequence
  source: /note="Description of Artificial Sequence: Synthetic peptide with caspase recognition/cleavage sequence, e.g., for Caspase 3/7"
DEVDG

SEQ ID NO: 4 - protein, 8 aa, Artificial Sequence
  source: /note="Description of Artificial Sequence: Synthetic peptide with caspase recognition/cleavage sequence, e.g., for Caspase 3/7"
GDEVDGIK

SEQ ID NO: 5 - protein, 4 aa, Artificial Sequence
  source: /note="Description of Artificial Sequence: Synthetic peptide with caspase recognition/cleavage sequence"
  VARIANT (1)..(1): /replace="Tyr" or "Ile" or "Leu" or "Asp" or "Val"
  MOD_RES (3)..(3): Any amino acid
  MISC_FEATURE (1)..(4): /note="Variant residues given in the sequence have no preference with respect to those in the annotations for variant positions"
WEXD

SEQ ID NO: 6 - protein, 5 aa, Artificial Sequence
  source: /note="Description of Artificial Sequence: Synthetic peptide with caspase recognition/cleavage sequence"
  VARIANT (1)..(1): /replace="Leu"
  MOD_RES (4)..(4): Any amino acid
  MISC_FEATURE (1)..(5): /note="Variant residues given in the sequence have no preference with respect to those in the annotations for variant positions"
VDEXD

SEQ ID NO: 7 - protein, 4 aa, Artificial Sequence
  source: /note="Description of Artificial Sequence: Synthetic peptide with caspase recognition/cleavage sequence"
  MOD_RES (2)..(2): Any amino acid
DXVD

SEQ ID NO: 8 - protein, 5 aa, Artificial Sequence
  source: /note="Description of Artificial Sequence: Synthetic peptide with caspase recognition/cleavage sequence"
  VARIANT (2)..(2): /replace="Tyr" or "Ile" or "Leu" or "Val"
  MOD_RES (4)..(4): Any amino acid
  MISC_FEATURE (1)..(5): /note="Variant residues given in the sequence have no preference with respect to those in the annotations for variant positions"
DWEXD

SEQ ID NO: 9 - protein, 4 aa, Artificial Sequence
  source: /note="Description of Artificial Sequence: Synthetic peptide with caspase recognition/cleavage sequence, e.g., for Caspase 1/5"
WEHD

SEQ ID NO: 10 - protein, 4 aa, Artificial Sequence
  source: /note="Description of Artificial Sequence: Synthetic peptide with caspase recognition/cleavage sequence, e.g., for Caspase 1"
YVAD

SEQ ID NO: 11 - protein, 4 aa, Artificial Sequence
  source: /note="Description of Artificial Sequence: Synthetic peptide with caspase recognition/cleavage sequence, e.g., for Caspase 1"
YVHD

SEQ ID NO: 12 - protein, 5 aa, Artificial Sequence
  source: /note="Description of Artificial Sequence: Synthetic peptide with caspase recognition/cleavage sequence, e.g., for Caspase 2"
VDVAD

SEQ ID NO: 13 - protein, 4 aa, Artificial Sequence
  source: /note="Description of Artificial Sequence: Synthetic peptide with caspase recognition/cleavage sequence, e.g., for Caspase 8"
IETD

SEQ ID NO: 14 - protein, 4 aa, Artificial Sequence
  source: /note="Description of Artificial Sequence: Synthetic peptide with caspase recognition/cleavage sequence, e.g., for Caspase 6"
VEID

SEQ ID NO: 15 - protein, 4 aa, Artificial Sequence
  source: /note="Description of Artificial Sequence: Synthetic peptide with caspase recognition/cleavage sequence, e.g., for Caspase 4/9"
LEVD

SEQ ID NO: 16 - protein, 4 aa, Artificial Sequence
  source: /note="Description of Artificial Sequence: Synthetic peptide with caspase recognition/cleavage sequence, e.g., for Caspase 10"
AEVD

SEQ ID NO: 17 - protein, 5 aa, Artificial Sequence
  source: /note="Description of Artificial Sequence: Synthetic peptide with caspase recognition/cleavage sequence, e.g., for Caspase 8"
DIETD

SEQ ID NO: 18 - protein, 5 aa, Artificial Sequence
  source: /note="Description of Artificial Sequence: Synthetic peptide with caspase recognition/cleavage sequence, e.g., for Caspase 9"
DLEHD

SEQ ID NO: 19 - protein, 5 aa, Artificial Sequence
  source: /note="Description of Artificial Sequence: Synthetic peptide with caspase recognition/cleavage sequence, e.g., for Caspase 1"
DYVAD

SEQ ID NO: 20 - protein, 5 aa, Artificial Sequence
  source: /note="Description of Artificial Sequence: Synthetic peptide with caspase recognition/cleavage sequence"
  VARIANT (2)..(2): /replace="Tyr" or "Ile" or "Leu" or "Val"
  MOD_RES (4)..(4): Any amino acid
  MISC_FEATURE (1)..(5): /note="Variant residues given in the sequence have no preference with respect to those in the annotations for variant positions"
DWVXD

SEQ ID NO: 21 - protein, 205 aa, Artificial Sequence
  source: /note="Description of Artificial Sequence: Synthetic peptide with caspase recognition/cleavage sequence"
  MOD_RES (1)..(100): Any amino acid or not present
  MOD_RES (106)..(205): Any amino acid or not present
XXXXXXXXXXXXXXXXXXXXXXXXXXXXXXXXXXXXXXXXXXXXXXXXXXXXXXXXXXXXXXXXXXXXXXXXXXXXXXXXXXXXXXXXXXXXXXXXXXXXDEVDGXXXXXXXXXXXXXXXXXXXXXXXXXXXXXXXXXXXXXXXXXXXXXXXXXXXXXXXXXXXXXXXXXXXXXXXXXXXXXXXXXXXXXXXXXXXXXXXXXXXX

SEQ ID NO: 22 - protein, 104 aa, Artificial Sequence
  source: /note="Description of Artificial Sequence: Synthetic cleaved peptide fragment after treatment with caspase"
  MOD_RES (1)..(100): Any amino acid or not present
XXXXXXXXXXXXXXXXXXXXXXXXXXXXXXXXXXXXXXXXXXXXXXXXXXXXXXXXXXXXXXXXXXXXXXXXXXXXXXXXXXXXXXXXXXXXXXXXXXXXDEVD

SEQ ID NO: 23 - protein, 101 aa, Artificial Sequence
  source: /note="Description of Artificial Sequence: Synthetic cleaved peptide fragment after treatment with caspase"
  MOD_RES (2)..(101): Any amino acid or not present
GXXXXXXXXXXXXXXXXXXXXXXXXXXXXXXXXXXXXXXXXXXXXXXXXXXXXXXXXXXXXXXXXXXXXXXXXXXXXXXXXXXXXXXXXXXXXXXXXXXXX

SEQ ID NO: 24 - protein, 5 aa, Artificial Sequence
  source: /note="Description of Artificial Sequence: Synthetic peptide with caspase recognition/cleavage sequence"
  VARIANT (2)..(2): /replace="Tyr" or "Ile" or "Leu" or "Val" or "Asp"
  VARIANT (3)..(3): /replace="Val"
  MOD_RES (4)..(4): Any amino acid
  MISC_FEATURE (1)..(5): /note="Variant residues given in the sequence have no preference with respect to those in the annotations for variant positions"
DWEXD